European Patent Specification EP 3 465 217 B1, published September 3, 2025. Title: RD33382PC. Applicant: Roche Diagnostic GmbH F.Hoffmann-La Roche AG Roche Diagnostics Operations, Inc. The sequence listing filed with the application follows.

SEQUENCE LISTING (2 sequences)

SEQ ID NO: 1 - protein, 191 aa, Hepatitis C virus
MSTNPKPQKKNKRNTNRRPQDVKFPGGGQIVGGVYLLPRRGPRLGVRATRKTSERSQPRGRRQPIPKARRPEGRTWAQPGYPWPLYGNEGCGWAGWLLSPRGSRPSWGPTDPRRRSRNLGKVIDTLTCGFADLMGYIPLVGAPLGGAARALAHGVRVLEDGVNYATGNLPGCSFSIFLLALLSCLTVPASA

SEQ ID NO: 2 - protein, 177 aa, Hepatitis C virus
MSTNPKPQKKNKRNTNRRPQDVKFPGGGQIVGGVYLLPRRGPRLGVRATRKTSERSQPRGRRQPIPKARRPEGRTWAQPGYPWPLYGNEGCGWAGWLLSPRGSRPSWGPTDPRRRSRNLGKVIDTLTCGFADLMGYIPLVGAPLGGAARALAHGVRVLEDGVNYATGNLPGCSFSIF